European Patent Specification EP 3 770 261 B1, published March 27, 2024. Title: NUCLEIC ACID MOLECULES AND APPLICATIONS THEREOF IN PREPARING HUMAN SINGLE-DOMAIN ANTIBODY. Applicant: CHONGQING JINMAIBO BIOTEC CO., LTD. The sequence listing filed with the application follows.

SEQUENCE LISTING (3 sequences)

SEQ ID NO: 1 - DNA, 15999 bp, Artificial Sequence
  The sequence is synthetized.
  misc_feature (1)..(8): Not1 restriction site (synthetic sequence)
  misc_feature (9)..(370): Homologous arm (human sequence)
  misc_feature (433)..(1444): Mouse IgH 5' enhancer (mouse sequence).
  misc_feature (3278)..(8527): mouse Igγ1 conversion element (Sγ1) (mouse sequence).
  misc_feature (8648)..(8692): Human Igγ1 Hinge (human sequence)
  misc_feature (8811)..(9141): Human Ig  γ1 CH2 (human sequence).
  misc_feature (9238)..(9560): Human Ig γ1 CH3 (human sequence).
  misc_feature (10862)..(10992): Mouse TM1 (mouse sequence).
  misc_feature (11810)..(11890): Mouse TM2 (mouse sequence).
  misc_feature (12611)..(13477): Mouse PolyA signal sequence (mouse sequence).
  misc_feature (13837)..(13870): Lox (synthetic sequence).
  misc_feature (13871)..(15192): pGK-Puromycin screening genes (synthetic sequences).
  misc_feature (15193)..(15226): Lox (synthetic sequence).
  misc_feature (15227)..(15508): Homologous arm (homologous recombination for linking to mouse 3'-LCR) (mouse sequence).
  misc_feature (15509)..(15516): AsiSI (synthetic sequence).
  misc_feature (15517)..(15991): Homologous arm (homologous recombination for linking to human Ig C-region sequence) (human sequence).
  misc_feature (15992)..(15999): Not1 (synthetic sequence)
gcggccgccgagatgcctgaacaaaccaggggtcttagtgatggctgaggaatgtgtctcaggagcggtgtctgtaggactgcaagatcgctgcacagcagcgaatcgtgaaatattttctttagaattatgaggtgcgctgtgtgtcaacctgcatcttaaattctttattggctggaaagagaactgtcggagtgggtgaatccagccaggagggacgcgtagccccggtcttgatgagagcagggttgggggcaggggtagcccagaaacggtggctgccgtcctgacaggggcttagggaggctccaggacctcagtgccttgaagctggtttccaagagaaaaggattgtttatcttaggaggcatcttagtgattgagtcaagggagaaaggcatctagcctcggtctcaaaagggtagttgctgtctagagaggtctggtggagcctgcaaaagtccagctttcaaaggaacacagaagtatgtgtatggaatattagaagatgttgcttttactcttaagttggttcctaggaaaaatagttaaatactgtgactttaaaatgtgagagggttttcaagtactcatttttttaaatgtccaaaattcttgtcaatcagtttgaggtcttgtttgtgtagaactgatattacttaaagtttaaccgaggaatgggagtgaggctctctcataacctattcagaactgacttttaacaataataaattaagtttcaaatatttttaaatgaattgagcaatgttgagttggagtcaagatggccgatcagaaccagaacacctgcagcagctggcaggaagcaggtcatgtggcaaggctatttggggaagggaaaataaaaccactaggtaaacttgtagctgtggtttgaagaagtggttttgaaacactctgtccagccccaccaaaccgaaagtccaggctgagcaaaacaccacctgggtaatttgcatttctaaaataagttgaggattcagccgaaactggagaggtcctcttttaacttattgagttcaaccttttaattttagcttgagtagttctagtttccccaaacttaagtttatcgacttctaaaatgtatttagaattcattttcaaaattaggttatgtaagaaattgaaggactttagtgtctttaatttctaatatatttagaaaacttcttaaaattactctattattcttccctctgattattggtctccattcaattcttttccaatacccgaagcatttacagtgactttgttcatgatcttttttagttgtttgttttgccttactattaagactttgacattctggtcaaaacggcttcacaaatctttttcaagaccactttctgagtattcattttaggagaaagactttttttttaaatgaatgcaattatctagacttatttcagttgaacatgctggttggtggttgagaggacactcagtcagtcagtgacgtgaagggcttctaagccagtccacatgctctgtgtgaactccctctggccctgcttattgttgaatgggccaaaggtctgagaccaggctgctgctgggtaggcctggactttgggtctcccacccagacctgggaatgtatggttgtggcttctgccacccatccacctggctgctcatggaccagccagcctcggtggctttgaaggaacaattccacacaaagactctggacctctccgaaaccaggcaccgcaaatggtaagccagaggcagccacagctgtggctgctgctcttaaagcttgtaaactgtttctgcttaagagggactgagtcttcagtcattgctttagggggagaaagagacatttgtgtgtcttttgagtaccgttgtctgggtcactcacatttaactttccttgaaaaactagtaaaagaaaaatgttgcctgttaaccaataatcatagagctcatggtactttgaggaaatcttagaaagcgtgtatagaaagtagggactctggggtcccaggttcaatcccagcattgttattacagtaactaagggaacagaagcaactctggattgaaggagggaaagacaagtagagggaagcccaagctgctctgagggactcagggtatgtgggggatccagagagccaggggaactcgagagctcaggacagaagactgagcacctgcaaaagagctgaggctggtaagagtaacaaggtaacctgggtaacaggttcagcagctccaggggagccaggagagatggaagtgtggggagccaggcagagcagctccatgacagccaggacaggtggaagtgtggtacccaggcagagcagctccatgacagccaggacaggtggaattgtggtgacccaggcagagcagctccagggcagccaggacaggtggaagtgtggtgacccaggcagagcatctataggggagccaggacaggtgggagtgtggtgacccaggcagagcagctccagggcatccaggacaggtggaattgtggtgacccaggcagagcagctacaggggagccaggaaaggtgggagtgtggtgacccaggcagagcagctacaggggagccaggacaggtgggagtgtggtgacccaggcagagcagctatagggcagccaggacaggtggaagtgtggtgacccaggcagagcagctacaggggagccaggaaaggtgggagtgtggtgacccaggcagagcagctacaggggagccaggaaaggtgggagtgtggtgacccaggcagagcagctacaggggagccaggaaaggtgggagtgtggtgacccaggcagagcagctacagggcagccaggacaggtggaagtgtggtgacccaggcagagcagctccatggcacccaggacaggtggaagtgtggtgacccaggcagagtagctacagggcagccaggacaggtggaagtgtggtgacccaggcagagcagcttcagggcagccaggacaggtggaagtgtggtgacccaggcagagcagcttcagggcagccaggacaggtggaagtgtggtgacccaggcagagcagcttcagggcagccaggacaggtgggagtgtggtgacccaggcagagcagctccaggggagccaggacaggtgggagtgtggtgacccaggcagagcagctccagggcagccaggacaggtggaagtgttgtgacccaggcagagcatctatagggtagccaggacaggtggaattgtggtgacccaggcagagcagctccagggcagccaggacaggtgggagtgtggtgacccaggcagagcatctataggggagccaggacaggtggaagtgtggtgacccaggcagagtagctacagggagccaggacaggtggaagtgtggtgacccaggcagagtagctcttggggagcctggacaggtgggagtgtggtgacccaggcagagcagctacaggggagctaggacaggtggaagtgtggtgacccaggcagagtagctcttggggagccaggacaggtggaagtgtggtgacccaggcagagcatctataggggagccaggacaggtgggagtgtggggatccaggtaaggcaggactggggagccaggacaggtggaagtgtggtgacccaggcagagcagctccagggcagccaggacaggtggaagtgtggtgacccaggcagagcagctccatggcagccaggacaggtggaaatgtggtgacccaggcagagcagctccagggcagccaggacaggtggaagtgtggtgacccaggcagagcatctataggggagccaggacaggtgggagtgtggtgacccaggcagagcagctccatggcagccaggacaggtgggagtgtggtgacccaggcagagcagctcatggcagccaggacaggtgggagtgtggtgacccagtcagagcagctgcagggcagccaggacaggtgggagtgtggtgacccaggcagagcatctataggggaaccaggacaggtggaagtgtggtgacccaggcagagcagctgcagggcagccaggacaggtgggagtgtggtgacccaggcagagcatctataggggaaccaggacaggtggaagtgtggtgacccaggcagagcagctatagggagccaggacaggtggaagtgtgttgatccagacaaaacacctacaggggagacaaatcagctagattgggcggatcctggcagatcagcttcaggggacctaggcaagtggaactgtggggacccgtgtagggcagctgtagggaaatcaggacaggtacaagtgtgtggatccatgcagtgtagtgccttgggagcctgaacagatagaagggtggggatacaggcagggtagctatagggaatccagttgaggtggaagaatggggatccaggcagagtagctatagggcagccaggagaaatggaagaatgcagatccaaacagaagagctacagaggagccaagacaactagaagtgtgtgaatccaggcagagcagtgccttaggagcaaggacagggaagctatagggaaaccaggacaggtggaagaatggggatccaggtgctgcagctacaggtaagcagggacaggtggaagtgtggagacccaggcagagcagctatagggcagccaggacaggtgggagtgtggggatccaggtaaggcaggactggggagtcaaggtaggtggaatgtgaagttccaggcagaacaggtccagggtgccaggacaggtacaagtttagtagttatagaggaacaggggcaggttagaatgaaggatgggcatcccgggtgagcaaatacaagggaactgatggcaaatggaagggcagggacccagactaaatggctacagagaagctgaggcaggtaagagtgtgggaacccagtcaaaaaccacagaagagcaggagctaattggcacgggctggggtgcatgctggctactcatagggaagctgggataagtagtagttggggattctaagcagtcacagagaagctgatcccggtgagagtacggggtacacagctgagcaaatactacatagctggagctgatggctgtataaggtaccaggctgagcagctgaaggtaacctggacctagtgggggtgtgggagacctggctgagcagctaccaaggatcagggatagacatgtaagcagtcaagctcagctactacatgagagctggagctagtatgaaggtggaggtccagttgagtgtctttagagaaactgaggcaagtgggagtgcagagatccaggctgagcagctccagcttagctggtataggtgacaggatgggggataacaaggctaagaacacacagagagcaggatctcctgggtaggttacaggtcaagactgagtagaatcaggggagctgaggttgggagtaatgcagaattccagacttagcagtccaggcaaactaaaccaagtgggagtgtgggagtcctaactgaacaaataccaggcatatgaagctgataagtgtgtataaagtaccaagctgagcagctacaggagagctgggatagctatgtggggagaccaggttaagcaaacagtggagagcaagataaagtcttaatgtatgcatccaggctgaatagacacaggggagctgaggaaggcagtactagaggattctaggcttagaagtcacagggaaactgaggcctgggtgagggtgggcatcctagctggaaaaatcaccagggagctggagctgatgggtataaaaaggtaccaggttgagcagctacaggagagctaggacatgtggggatgttttgttccaggctgaacaactgtagagcatcagggggaggtggaactttaagaagtcaggctgagcagctacaggagagctgcagctattcggtatgtggaggtccagccagagcagttacagggtagctgggataaatggggctggagaaccaggctaagaagacacaggggagcaggttctagtctgcataggagtggggatccaggtcgagtacacacagaagagaaaagggtaggtagtaatggaggattctagactcagctataactgagtggtagtgtgagtgttctagctggaaaaaaaaataccatgaagctggagctgatgggtataaaaggaacgagcctgagaaactgtagggtatctggggtggatggggatgtggggagtcatgctgagctgctacaagggcagtgtggcctctaggagtgtaggggaccaaactgagcatctacagggaaactgaggcaaactggagtgtagggctccagaatgagcaactgcaggtcagctgaggccggtaagagtgtggggaaccagactggacagttagttgcaagttagccagggtaggtgagagttctattagagaagcctcagcagaatgggaagtgggaactaggaaaccaggatgagcacctaacaacagaagtgaggcaggttagggtgtaggggatgagctgtgcagctactgtggagcacgcagactggaatagaagaggttctggctgaacacttgaagggaaccaggtaggcaggaggcagtgtgtacagacagctgaatgagacatcatgcagggccagttccctgccctgagctacattagctgggaccagggccagcggttgaggaaccaggcagaggtaaaatggtggtgtgataggaagccaatggcagaggggagggagaagttatgcttatgtcatgctggaatgtaggaaggggaaagagccaggatgtctaggctggagctgatccggctgtctgctctgatggcagcaacaggcctgagcttctctggactcaagaagccagggcaacaaaataaagggggcctagcagagcaaagacactgctagcactgggatcaggaaaacaggacaagactcccgatccaggaggtcatgggagggaaggagaagactacaggggactgtccttgggaaagagtaagggcccactggagggagtgctcaggaagcaagcccattgacaggggagaacaaggctggtggacgtctggatgggcagtaggcagccccaagtcccaggagggagagaagaggcagataggaaaacaggtcaggtctagcagaggcctactgaagtactctcctcaggacagaaccctgaatactggaaaatgcggaactgctgcaggcacaaagaatagctgaggtctaagagtaaaacagactaggggatgagaggaccttaggaagagcctttggctgagcaggaacaagaacaggggaaatcctagggctgacattgccagtggaaacatacaggctggagctctttagtcaggagctccagctgtgatctagacatcaggcaggaagatcaaatctgtcccaacaatacaggggacagaggctcaacctagagtgtgagcatcaggggctgtgcaggagatttcagagctcaggtgcagcagagactagcatggccctggggataaagggaaggatccaagggacaaggggataatcctggggaggtaagggccagcttcgtgacagaaggtggtggtgtccaacttcaagagccctgtgctacaatttaaaaaaaaaaaaaaaggaaagggacttctctgtgtttggcaacacaagtgcgatgcacaggcaggaagatcaaatctgtcccaacaatacaggggacagagggtcaacctacaaaaggaaagaacctggggcagtgtgaagacaacactgtagaagccaaggctgagttcactgagctctcgttagtgagactacacagcaaggaggtggcgggcactgagcagtgaggccccgggaagtgggggtgatggtggtgacggtggtaactgttaagaactgggggaaagaattgtggagaaccaagctaaatagttatgtcaaaccacatgtttaggagcctgggttgacttcatagggagtaggcatggaggctaatctagaggtttgtgtataggcaagaagtgaatcctgacccaagaatagagagtgctaaacggacttagttcaaagacaactgaaaaagacaatgcctgcaaaacaaagctaaggccagagctcttggactatgaagagttcagggaacctaagaacagggaccatctgtgtacaggccaaggccggtagaagcagcctaggaagtgtcaagagccaacgtggctgggtgggcaaagacaggaagggactgttaggctgcagggatgtgccgacttcaatgtgcttcagtattgtccagattgtgtgcagccatatggcccaggtataagaggtttaacagtggaacacagatgcccacatcagacagctggggggcgggggtgaacacagatacccatactggaaagcaggtggggcattttcctaggaacgggactgggctcaatggcctcaggtctcatctggtctggtgatcctgacattgataggcccaaatgttggatatcacctactccatgtagagagtcggggacatgggaagggtgcaaaagagcggccttctagaaggtttggtcctgtcctgtcctgtctgacagtgtaatcacatatactttttcttgtagagcccaaatcttgtgacaaaactcacacatgcccaccgtgcccaggtaagccagcccaggcctcgccctccagctcaaggcgggacaggtgccctagagtagcctgcatccagggacaggccccagccgggtgctgacacgtccacctccatctcttcctcagcacctgaactcctggggggaccgtcagtcttcctcttccccccaaaacccaaggacaccctcatgatctcccggacccctgaggtcacatgcgtggtggtggacgtgagccacgaagaccctgaggtcaagttcaactggtacgtggacggcgtggaggtgcataatgccaagacaaagccgcgggaggagcagtacaacagcacgtaccgtgtggtcagcgtcctcaccgtcctgcaccaggactggctgaatggcaaggagtacaagtgcaaggtctccaacaaagccctcccagcccccatcgagaaaaccatctccaaagccaaaggtgggacccgtggggtgcgagggccacatggacagaggccggctcggcccaccctctgccctgagagtgaccgctgtaccaacctctgtccctacagggcagccccgagaaccacaggtgtacaccctgcccccatcccgggatgagctgaccaagaaccaggtcagcctgacctgcctggtcaaaggcttctatcccagcgacatcgccgtggagtgggagagcaatgggcagccggagaacaactacaagaccacgcctcccgtgctggactccgacggctccttcttcctctacagcaagctcaccgtggacaagagcaggtggcagcaggggaacgtcttctcatgctccgtgatgcatgaggctctgcacaaccactacacacagaagagcctctccctgtctccgggtaaatgataatgtcctggtgatttctgagatgtagagtctagctaggtcatggaatgaggggtctccatggtttgaggcctgagttgtgactaaggaaaaacccataggcctacactgccacacccagcacttttgaatttgcctgacatgaaaagaatttacctctccctggaaagtggagccttatccctaggcagttcccttaccagaccttcctctagcttgcactttgttctgggcacagaatgtgtctaaccccccaaagcaaggaagacacaacctctacctccctcactctgtccttaccccttttcctggctaagcatctcactgagtgcgctgaatagatgcatgtggccacagtcttgcagacagacccttgccatctctccactcagctttccagaggctaagtctagcccgtatggtgataatgcagggagctctatgctatctcagtgctatcagactcccaagtggaggatgaacatggacccattaaaaccaacctgcgcagcaacaccctgccaataaggcccgtatgtgaaaatgtgcacacatctacacatgcacaggcacacacacacacacatgcatgggcacacacacatacagagagagagaatcacagaaactcccatgagcatcctatacagtactcaaagataaaaaggtaccaggtctacccacatgatcatcctcggcatttacaagtgggccaactgatacagataaaacttttctatgccaaggacgccaacatatacacaagtccgctcatgacaaatctgtccctgaacctcagactggcgcccgtgactcatacagtggacactcctccaaagctgtatagcttcctttacttccctgtgtgtactttctctgaagtacactcatcacacagaagaggccctgtgattactctggccctctgttcttggtcatcagagaatagacagaagatcaggcaaactacacagacacttcccacaatcatcacaggccctgactctgctctccagtctcaaaactgaaggctggagcacacagaataagctcctgcacaggccaggccagtatcgggtccagtgtgtctgactgagcccagggacaaaatggcagcactttggggaactgaggtttctggtccaagaaggagagatggaggcccagggagggtctgctgacccagcccagcccagcccagctgcagctttctcctgggcctccatacagcctcctgccacacagggaatggccctagccccaccttattgggacaaacactgaccgccctctctgtccagggctgcaactggacgagacctgtgctgaggcccaggacggggagctggacgggctctggacgaccatcaccatcttcatcagcctcttcctgctcagtgtgtgctacagcgctgctgtcacactcttcaaggtcagccatactgtccccacagtgtctacaatgtcctcatactcttccccatactgtccctgtggtgacctataccccacactgtcccatgctaatgaccacagtcttacatgctatgtaatgctgtctacccttctgtatgcacagtctcacaatgtcccatgcagtctccacgatgctccatactgtccccattccaacccatgctgccccttgttccccgctatgctgtcccatgctattgtctgtattttcatgctcttttcacactgtccctagtgtcacattctgcccatgttgtccaccacattgtccccactctgtacacagcctcacactgtaccctgctacccgataatgttccctgttgtccccaactctctccctgcaccatttgtcaactgtcccctgaattcccatgttgttcccacactgttagtgtgtaatgtgctctgtcccaggtgtaccttgttccgtgctgtctcacttcatcgcccattctgtccttgtactaaccccactctatcaccacactgtccctatgcactgcccacattgtcctcatactgtcccattttgtatcttcatcctgtccccatagtgtccaatgatctaccccacactattcccacttcatgcccctacaatttccctattccattcctctctggtcaccatgccatccttcccactcctgcacagctggagagggactcccgggatgagtccttgcccagatgagctacctatctagaggagtcttcaggtgggaagggaatgcagtcttgatcttggtcttattcaccctgtctcacaggtaaagtggatcttctcctcggtggtggagctgaagcagacactggttcctgaatacaagaacatgattgggcaagcaccctaggccacctcctgtaatggcatttcccaggccccgaaggaccctgtccaatatgccaagcagcacaactgagatcacactgtctgctcatctcgctttcctccgaccccgagactcagctactctcaaattttccctctctgaaggaccatgtggacattacattgctccaggccacagccaccaggacctaaaacaccatcacagcagcaccaaagacactggatagacccacaagggcaatagtttcctcaacagtatatccaaactgttgggacaaacgagcaatcactgaagaagtgacaagttcccacaatgtcagtgtccagctgagaagggacaaaaagtggtaccagccctgtccacaccaccttctaattcacaggaatacgtgatagaagaggcaggttgtagatccgaaagatgagacagattttatcaactccagaaagagctgggtccaactgaattattctagcgaccttggcattgtcatgacctgccatgaccttcctccttaacacttcgataaaccctgggatatggaaaatgcctgtgtttctcagggtttgggaaagaaccatccatgttgggattcttgtgtagatcctccttctggtcacagatgcaatacactggattttcaggcaaaggagcaaattcacagacaactctggccctacagccctaagacctagacaccaccatctccttggaattatcaaatttaacacccggcacacaacaaagaaggactgggactttgaggcctttgtgtagccctagagggggcagaggccactgagcagggattgggtgatcacaaggacctcctggagagggacctgaggagcaggttccaattgggccaaagaaagaagaacaacaatagagatgaaggatgctggaaagagccatggtacagcagtcttgtccttcagacatgactcttacagcccaggactcttacagtagctagctggagcagaagtccaagggattaccatgccctagggccacaggctactggagggtggagtgagtctactacacaggtccaatgcctgtttctccattgcttctcagccaatgagaaatcagagtctccacctccaagaaaaaggaaggtggaaatgaaaggtgagcacctgccttcccgtgactggcagaaagatctccacggactcaaggctttgacttcaaacttcccgtagatccctgatgtctttaaggactctgtctgctttgttggttttgtttgtttgttttgtactttgtcaataaaacatttttcaaatattctacaattgctgtgctcttcctatgcaaactggccctggcacttcaaaacatggcacagttaagttgaccagtgggccatgcagagcatactacccctcctggtcctgtgtcctaccagatatcctctaagtgtcccttcactgctgggctccagttctgctgccctgaaccacacaggtcctcagtctgtcctccctatgggcagtttcatcccagccagaagctgccctgtggcccctaggctgcccaggcatggtctcccacaccaaccacacaaactaagaagcctgtcccatacattgacctcaggctcagtgataacatttctatagaaaaaggaaaggaataagaaaaaaaaaactccatattacatgggggctgcctaccttgctgatgcttattgtctcaagcaagtttggagaagttccaaatcaggcactgacagggtgggttctcagccatgctcttcttacctggtaggtgccttctcccccatggcacctcacaggctctccatctgtgtgtgtctgggtcctgatctcttctcataagtacaaagtcaggctggaagaggtacaccctagccctcattataacttaccagtttatgatcctgtctgcaaacatctgaggtccctgtggctataacttcgtataatgtatgctatacgaagttatctaccgggtaggggaggcgcttttcccaaggcagtctggagcatgcgctttagcagccccgctgggcacttggcgctacacaagtggcctctggctcgcacacattccacatccaccggtaggcgccaaccggctccgttctttggtggccccttcgcgccaccttctactcctcccctagtcaggaagttcccccccgccccgcagctcgcgtcgtgcaggacgtgacaaatggaagtagcacgtctcactagtctcgtgcagatggacagcaccgctgagcaatggaagcgggtaggcctttggggcagcggccaatagcagctttgctccttcgctttctgggctcagaggctgggaaggggtgggtccgggggcgggctcaggggcgggctcaggggcggggcgggcgcccgaaggtcctccggaggcccggcattctgcacgcttcaaaagcgcacgtctgccgcgctgttctcctcttcctcatctccgggcctttcgacctgcagcagcacgtgttgacaattaatcatcggcatagtatatcggcatagtataatacgacaaggtgaggaactaaaccatgaccgagtacaagcccacggtgcgcctcgccacccgcgacgacgtcccccgggccgtacgcaccctcgccgccgcgttcgccgactaccccgccacgcgccacaccgtcgacccggaccgccacatcgagcgggtcaccgagctgcaagaactcttcctcacgcgcgtcgggctcgacatcggcaaggtgtgggtcgcggacgacggcgccgcggtggcggtctggaccacgccggagagcgtcgaagcgggggcggtgttcgccgagatcggcccgcgcatggccgagttgagcggttcccggctggccgcgcagcaacagatggaaggcctcctggcgccgcaccggcccaaggagcccgcgtggttcctggccaccgtcggcgtctcgcccgaccaccagggcaagggtctgggcagcgccgtcgtgctccccggagtggaggcggccgagcgcgccggggtgcccgccttcctggagacctccgcgccccgcaacctccccttctacgagcggctcggcttcaccgtcaccgccgacgtcgaggtgcccgaaggaccgcgcacctggtgcatgacccgcaagcccggtgcctgagcgggactctggggttcgaataaagaccgaccaagcgacgtctgagagctccctggcgaattcggtaccaataaaagagctttattttcatgatctgtgtgttggtttttgtgtgcggcgcgccgtttaaacgcggataacttcgtataatgtatgctatacgaagttatagaccgacgtgacaacttcccagcccactcacagactttcctgagcaataaattgatgcaaaaccacaaattcctactctcaaaaacaaacattaacaaaggattgggggagggggtcaggggtagtatggtggcgttgggcagggtaaactcagggtacccattgtctaatgtctgagacataacttgaacatatgtgtagctgcagccaaagatgaacaagtgatggtatttgtgtcctcttcagacccgataccaggtcattaagcttgagatctggacgcgatcgccagcctccagaatggtgggaaataagtttctgttgtttctcagccaccacgtctgtagtatgtggaagtcatcagaatcaaaattgagtcacctgtggttttttttttttctaaatccctgacaaatagagcctaggaaggccaagaagagaagagggttctcatccataaacacttgataacaaaaactatcaccaaggactctacaaaaactgcaactggcacaaagaccatcacaaccttacacagaaagtacttctgtgaggacatcttcccagcaacgggctgtccaacctcagactggcattgcctttgttattggtccttgtagagagggtaattatctcaaagcaatcatgtaatcctcctcatttttcctttgaaagccttggtctccctttgcctccctgaatacgcacatagctgatcatggcaggtgtatcccactgcagtgctctacctccaaatagatatcgcggccgc

SEQ ID NO: 2 - DNA, 11862 bp, Artificial Sequence
  The sequence is synthetized.
  misc_feature (1)..(8): Not1 restriction site (synthetic sequence).
  misc_feature (9)..(370): Homologous arm (human sequence).
  misc_feature (433)..(1444): Mouse IgH 5' enhancer (mouse sequence).
  misc_feature (2550)..(4451): Mouse IgM conversion element (Sμ) (mouse sequence).
  misc_feature (5674)..(6012): Mouse IgM CH2 (mouse sequence).
  misc_feature (6292)..(6609): Mouse IgM CH3 (mouse sequence).
  misc_feature (6717)..(7111): Mouse IgM CH4 (mouse sequence).
  misc_feature (7112)..(7341): Mouse PolyA signal sequence (mouse sequence).
  misc_feature (8910)..(9025): Mouse TM1 (mouse sequence).
  misc_feature (9144)..(9149): Mouse TM2 (mouse sequence).
  misc_feature (9265)..(9556): Mouse PolyA signal sequence (mouse sequence).
  misc_feature (9700)..(9733): Lox (synthetic sequence).
  misc_feature (9734)..(11055): pGK-Puromycin screening gene (synthetic sequence).
  misc_feature (11056)..(11089): Lox (synthetic sequence).
  misc_feature (11090)..((11371): Homologous arm (homologous recombination for linking to mouse Ig γ1 Sγ1) (mouse sequence).
  misc_feature (11372)..(11379): AsiSI (synthetic sequence).
  misc_feature (11380)..(11854): Homologous arm (homologous recombination for linking to human Ig C-region sequence) (human sequence).
  misc_feature (11855)..(11862): Not1 (synthetic sequence).
gcggccgccgagatgcctgaacaaaccaggggtcttagtgatggctgaggaatgtgtctcaggagcggtgtctgtaggactgcaagatcgctgcacagcagcgaatcgtgaaatattttctttagaattatgaggtgcgctgtgtgtcaacctgcatcttaaattctttattggctggaaagagaactgtcggagtgggtgaatccagccaggagggacgcgtagccccggtcttgatgagagcagggttgggggcaggggtagcccagaaacggtggctgccgtcctgacaggggcttagggaggctccaggacctcagtgccttgaagctggtttccaagagaaaaggattgtttatcttaggaggcatcttagtgattgagtcaagggagaaaggcatctagcctcggtctcaaaagggtagttgctgtctagagaggtctggtggagcctgcaaaagtccagctttcaaaggaacacagaagtatgtgtatggaatattagaagatgttgcttttactcttaagttggttcctaggaaaaatagttaaatactgtgactttaaaatgtgagagggttttcaagtactcatttttttaaatgtccaaaattcttgtcaatcagtttgaggtcttgtttgtgtagaactgatattacttaaagtttaaccgaggaatgggagtgaggctctctcataacctattcagaactgacttttaacaataataaattaagtttcaaatatttttaaatgaattgagcaatgttgagttggagtcaagatggccgatcagaaccagaacacctgcagcagctggcaggaagcaggtcatgtggcaaggctatttggggaagggaaaataaaaccactaggtaaacttgtagctgtggtttgaagaagtggttttgaaacactctgtccagccccaccaaaccgaaagtccaggctgagcaaaacaccacctgggtaatttgcatttctaaaataagttgaggattcagccgaaactggagaggtcctcttttaacttattgagttcaaccttttaattttagcttgagtagttctagtttccccaaacttaagtttatcgacttctaaaatgtatttagaattcattttcaaaattaggttatgtaagaaattgaaggactttagtgtctttaatttctaatatatttagaaaacttcttaaaattactctattattcttccctctgattattggtctccattcaattcttttccaatacccgaagcatttacagtgactttgttcatgatcttttttagttgtttgttttgccttactattaagactttgacattctggtcaaaacggcttcacaaatctttttcaagaccactttctgagtattcattttaggagaaagactttttttttaaatgaatgcaattatctagacttatttcagttgaacatgctggttggtggttgagaggacactcagtcagtcagtgacgtgaagggcttctaagccagtccacatgctctgtgtgaactccctctggccctgcttattgttgaatgggccaaaggtctgagaccaggctgctgctgggtaggcctggactttgggtctcccacccagacctgggaatgtatggttgtggcttctgccacccatccacctggctgctcatggaccagccagcctcggtggctttgaaggaacaattccacacaaagactctggacctctccgaaaccaggcaccgcaaatggtaagccagaggcagccacagctgtggctgctgctcttaaagcttgtaaactgtttctgcttaagagggactgagtcttcagtcattgctttagggggagaaagagacatttgtgtgtcttttgagtaccgttgtctgggtcactcacatttaactttccttgaaaaactagtaaaagaaaaatgttgcctgttaaccaataatcatagagctcatggtactttgaggaaatcttagaaagcgtgtatacaattgtctggaattatttcagttaagtgtattagttgaggtactgatgctgtctctacttcagttatacatgtgggtttgaattttgaatctattctggctcttcttaagcagaaaatttagataaaatggatacctcagtggtttttaatggtgggtttaatatagaaggaatttaaattggaagctaatttagaatcagtaaggagggacccaggctaagaaggcaatcctgggattctggaagaaaagatgtttttagtttttatagaaaacactactacattcttgatctacaactcaatgtggtttaatgaatttgaagttgccagtaaatgtacttcctggttgttaaagaatggtatcaaaggacagtgcttagatccgaggtgagtgtgagaggacaggggctggggtatggatacgcagaaggaaggccacagctgtacagaattgagaaagaatagagacctgcagttgaggccagcaggtcggctggactaactctccagccacagtaatgacccagacagagaaagccagactcataaagcttgctgagcaaaattaagggaacaaggttgagagccctagtaagcgaggctctaaaaagcacagctgagctgagatgggtgggcttctctgagtgcttctaaaatgcgctaaactgaggtgattactctgaggtaagcaaagctgggcttgagccaaaatgaagtagactgtaatgaactggaatgagctgggccgctaagctaaactaggctggcttaaccgagatgagccaaactggaatgaacttcattaatctaggttgaatagagctaaactctactgcctacactggactgttctgagctgagatgagctggggtgagctcagctatgctacgctgtgttggggtgagctgatctgaaatgagatactctggagtagctgagatggggtgagatggggtgagctgagctgggctgagctagactgagctgagctagggtgagctgagctgggtgagctgagctaagctggggtgagctgagctgagcttggctgagctagggtgagctgggctgagctggggtgagctgagctgagctggggtaagctgggatgagctggggtgagctgagctgagctggagtgagctgagctgggctgagctggggtgagctgggctgagctgggctgagctgggctgagctggggtgagctgagctggggtgagctgagctgagctggggtgagctgagctgagctggggtgagctggggtgagctgagctggggtgagctgagctgagctggggtgagctgagctggggtgagctgagctgagctggggtgagctgagctgagctgagctgagctgagctggggtgagctgagctgagctgagctggggtgagctggggtgagctgagctgagctggagtgagctgagctgggctgagctggggtgagctgggctgagctggggtgagctgagctgagctgagctgagctggggtgagctgagctgagctggggtgagctgagctggggtgagctgggctgagctgagctgagctgagctgagctgagctgagctgagctgagctgagctgagctgagctgagctgagctgagctgagctgagctggggtgagctgagctgagctgggctgagctggggtgagctgggctgagctgggctgagctgggctgagctggggtgagctgagctggggtgagctgagctgagctgggctgagctgagctgagctggggtgagctgagctgagctggggtgagctgagctgagctgagctggggtgagctgagctgggctgagcagggctgagctggggtgagctgagctgagctggggtgagctgggctgagctgggctgagctgagctgagctgggctgagctgggctgagctgggctgagctgggctgagctgggctgagctggggtgagctgagctgagctggggtgagctggggtgagctgagctggggtgagctgagctggggtgagctgagctgagctggggtgagctgagctggggtgagctgagctgagctggggtgagctgagctgagctggggtgagctgagctagggtgaactgggctgggtgagctggagtgagctgagctgaggtgaactggggtgagccgggatgttttgagttgagctggggtaagatgagctgaactggggtaaactgggatgagctgtggtgagcggagctggattgaactgagctgtgtgagctgagctggggtcagctgagcaagagtgagtagagctggctggccagaaccagaatcaattaggctaagtgagccagattgtgctgggatcagctgtactcagatgagctgggatgaggtaggctgggatgagctgggctagctgacatggattatgtgaggctgagctagcatgggctggcctagctgatgagctaagcttgaatgagcggggctgagctggactcagatgtgctagactgagctgtactggatgatctggtgtagggtgatctggactcaactgggctggctgatgggatgcgccaggttgaactaggctcagataagttaggctgagtagggcctggttgagatggttcgggatgagctgggaaaagatggactcggaccatgaactgggctgagctgggttgggagaccatgaattgagctgaactgagtgcagctgggataaactgggttgagctaagaatagactacctgaattgtgccaaactcggctgggatcaattggaaattatcaggatttagatgagccggactaaactatgctgagctggactggttggatgtgttgaactggcctgctgctgggctggcatagctgagttgaacttaaatgaggaaggctgagcaaggctagcctgcttgcatagagctgaactttagcctagcctgagctggaccagcctgagctgagtaggtctaaactgagttaaaaatcaacagggataatttaacagctaatttaacaagcctgaggtctgagattgaatgagcagagctgggatgaactgaatgagtttcaccaggcctggaccagttaggctaggacctcgttctatagaggcagactgtgtgctacagtggagtttcaagatgattccatgagtcctccccgcccccaacataacccaccttcctcctaccctacacgcctgtctggtgtgtaaatcccagctttgtgtgctgatacagaagcctgagcccctcccccacctccacctacctattactttgggatgagaatagttctcccagccagtgtctcagagggaagccaagcaggacaggcccaaggctacttgagaagccaggatctaggcctctccctgagaacgggtgttcatgcccctagagttggctgaagggccagatccacctactctagaggcatctctccctgtctgtgaaggcttccaaagtcacgttcctgtggctagaaggcagctccatagccctgctgcagtttcgtcctgtataccaggttcacctactaccatatctagccctgcctgccttaagagtagcaacaaggaaatagcagggtgtagagggatctcctgtctgacaggaggcaagaagacagattcttacccctccatttctcttttatccctctctggtcctcagctgtcgcagagatgaaccccaatgtaaatgtgttcgtcccaccacgggatggcttctctggccctgcaccacgcaagtctaaactcatctgcgaggccacgaacttcactccaaaaccgatcacagtatcctggctaaaggatgggaagctcgtggaatctggcttcaccacagatccggtgaccatcgagaacaaaggatccacaccccaaacctacaaggtcataagcacacttaccatctctgaaatcgactggctgaacctgaatgtgtacacctgccgtgtggatcacaggggtctcaccttcttgaagaacgtgtcctccacatgtgctgccagtgagtggcctgggctaagcccaatgcctagccctcccagattagggaagtcctcctacaattatggccaatgccacccagacatggtcatttgctccttgaactttggctccccagagtggccaaggacaagaatgagcaataggcagtagaggggtgagaatcagctggaaggaccagcatcttcccttaagtaggtttgggggatggagactaagcttttttccaacttcacaactagatatgtcataacctgacacagtgttctcttgactgcaggtccctccacagacatcctaaccttcaccatccccccctcctttgccgacatcttcctcagcaagtccgctaacctgacctgtctggtctcaaacctggcaacctatgaaaccctgaatatctcctgggcttctcaaagtggtgaaccactggaaaccaaaattaaaatcatggaaagccatcccaatggcaccttcagtgctaagggtgtggctagtgtttgtgtggaagactggaataacaggaaggaatttgtgtgtactgtgactcacagggatctgccttcaccacagaagaaattcatctcaaaacccaatggtaggtatccccccttcccttcccctccaattgcaggacccttcctgtacctcatagggagggcaggtcctcttccaccctatcctcactactgtcttcatttacagaggtgcacaaacatccacctgctgtgtacctgctgccaccagctcgtgagcaactgaacctgagggagtcagccacagtcacctgcctggtgaagggcttctctcctgcagacatcagtgtgcagtggcttcagagagggcaactcttgccccaagagaagtatgtgaccagtgccccgatgccagagcctggggccccaggcttctactttacccacagcatcctgactgtgacagaggaggaatggaactccggagagacctatacctgtgttgtaggccacgaggccctgccacacctggtgaccgagaggaccgtggacaagtccactggtaaacccacactgtacaatgtctccctgatcatgtctgacacaggcggcacctgctattgaccatgctagcgctcaaccaggcaggccctgggtgtccagttgctctgtgtatgcaaactaaccatgtcagagtgagatgttgcattttataaaaattagaaataaaaaaaatccattcaaacgtcactggttttgattatacaatgctcatgcctgctgagacagttgtgttttgcttgctctgcacacaccctgcatacttgcctccaccctggcccttcctctaccttgccagtttcctccttgtgtgtgaactcagtcaggcttacaacagacagagtatgaacatgcgattcctccagctacttctagatatatggctgaaagcttgcctaacctggtgcaggcagcattcaggcacatatatagacacacatgcatttatacatagatatataggtacacatgtgtagacacatacatgaatgtgtattcatggacacacagacaaaggtacacatatatacacatgagttcatgcgcacacacatgcatggacacttacaaacgccttcagagacaaataggcatagacacacaaccactcacagaaacagataccaatatgcatggtcctgtgtacacagaaacagactataggcaaatatacacaaataaactatatagatacaaagatatgcatatacacacatgtacagaaacatcttcacatgtgtacactaacatgtgaacaggtatagcacacagatacacctggactctgaccagggctgtaatctccaaggctcacggctcagagagcctacactaggctgggtcactgatactcctcaggagcccactctatgattgggagagataaccccaggtacaaagtatgcctatctgtctcaacaccatggggcagaagatactccactaaccacccatgacagaaagttagccttggctgtgtctccattaatagaacacctcagaagaccaatgtgaaattgcctaacccactcacacccaccctgatctccagttcaaaatgcagaaaacataatgcagttgtccaaaagatgccccaaccacacacacacacacacacacacacacacacacacacacacacacacacacacacacacaccatcaaggagcctctgtaaggagtcaccacccaataacactgcctctttgggctcatatcctggacattcttcatattcatatccatttggggcctaggctttagatatccccaagggctcatctttacagggatcagagatcccaataaatgccctggtcccacagcctccctcaggtatctgtctgtttatctcttggtaccaagacccaacattgctggcaggggtaggacaagcaacgcacgggaactctgatcaaagaaagtcatgagatgcctgagtccttcaggaagtaaggagggacaacctctggtatccctgttcttattgctaaagcccaagagacagggagacctgctctaaattctcagtctaaacagcaccgatggcaccacctgctcagggaaagtccagagcacaccaatatcattttgccacagttcctgagtctgcctttacccaggtccatacattgcatctgtcttgcttgctctgctgccccagggctcctggaacaaaggctccaaattagtgtgtcctacagcttggcctgttctgtgcctccgtctagcttgagctattaggggaccagtcaatactcgctaagattctccagaaccatcagggcaccccaacccttatgcaaatgctcagtcaccccaagacttggcttgaccctccctctctgtgtcccttcatagagggggaggtgaatgctgaggaggaaggctttgagaacctgtggaccactgcctccaccttcatcgtcctcttcctcctgagcctcttctacagcaccaccgtcaccctgttcaaggtagtgtggttgtggggctgaggacacagggctgggacagggagtcaccagtcctcactgcctctacctctactccctacaagtggacagcaattcacactgtctctgtcacctgcaggtgaaatgactctcagcatggaaggacagcagagaccaagagatcctcccacagggacactacctctgggcctgggatacctgactgtatgactagtaaacttattcttacgtctttcctgtgttgccctccagcttttatctctgagatggtcttctttctagactgaccaaagactttttgtcaacttgtacaatctgaagcaatgtctggcccacagacagctgagctgtaaacaaatgtcacatggaaataaatactttatcttgtgaactcactttattgtgaaggaatttgttttgtttttcaaacctttcctgcggtgttgacagcccaaggattatctgaatagagcttaggaactggaaatggaacagtgcagtctgatggtacttaagggagaaagagggaaaggaggtgtggaagaagaaaaaagagaagcagagggggaggggagaagggagagggagagggagagggagagggagagggagagggagagggagagagagagagagagagagagagagagagagagagagagagagcatgcactataacttcgtataatgtatgctatacgaagttatctaccgggtaggggaggcgcttttcccaaggcagtctggagcatgcgctttagcagccccgctgggcacttggcgctacacaagtggcctctggctcgcacacattccacatccaccggtaggcgccaaccggctccgttctttggtggccccttcgcgccaccttctactcctcccctagtcaggaagttcccccccgccccgcagctcgcgtcgtgcaggacgtgacaaatggaagtagcacgtctcactagtctcgtgcagatggacagcaccgctgagcaatggaagcgggtaggcctttggggcagcggccaatagcagctttgctccttcgctttctgggctcagaggctgggaaggggtgggtccgggggcgggctcaggggcgggctcaggggcggggcgggcgcccgaaggtcctccggaggcccggcattctgcacgcttcaaaagcgcacgtctgccgcgctgttctcctcttcctcatctccgggcctttcgacctgcagcagcacgtgttgacaattaatcatcggcatagtatatcggcatagtataatacgacaaggtgaggaactaaaccatgaccgagtacaagcccacggtgcgcctcgccacccgcgacgacgtcccccgggccgtacgcaccctcgccgccgcgttcgccgactaccccgccacgcgccacaccgtcgacccggaccgccacatcgagcgggtcaccgagctgcaagaactcttcctcacgcgcgtcgggctcgacatcggcaaggtgtgggtcgcggacgacggcgccgcggtggcggtctggaccacgccggagagcgtcgaagcgggggcggtgttcgccgagatcggcccgcgcatggccgagttgagcggttcccggctggccgcgcagcaacagatggaaggcctcctggcgccgcaccggcccaaggagcccgcgtggttcctggccaccgtcggcgtctcgcccgaccaccagggcaagggtctgggcagcgccgtcgtgctccccggagtggaggcggccgagcgcgccggggtgcccgccttcctggagacctccgcgccccgcaacctccccttctacgagcggctcggcttcaccgtcaccgccgacgtcgaggtgcccgaaggaccgcgcacctggtgcatgacccgcaagcccggtgcctgagcgggactctggggttcgaataaagaccgaccaagcgacgtctgagagctccctggcgaattcggtaccaataaaagagctttattttcatgatctgtgtgttggtttttgtgtgcggcgcgccgtttaaacgcggataacttcgtataatgtatgctatacgaagttatatgacatcttgttgtggaatagcaaacagagaagactgtttggacatcgatttaaggcaatagaaagtctttactagccaacctgtgactacactgggtgttcaggatctcagtgtagccctgaacctttctcagggtgagattttaggtaaaaattatgttctgggttgacatagttcagttaacaagaacacttagccagaaacagaactacaagacccaaaaagcaaagttaaaacatttacaaactttcctagaactgtatgaactttaatggattaggcgatcgccagcctccagaatggtgggaaataagtttctgttgtttctcagccaccacgtctgtagtatgtggaagtcatcagaatcaaaattgagtcacctgtggttttttttttttctaaatccctgacaaatagagcctaggaaggccaagaagagaagagggttctcatccataaacacttgataacaaaaactatcaccaaggactctacaaaaactgcaactggcacaaagaccatcacaaccttacacagaaagtacttctgtgaggacatcttcccagcaacgggctgtccaacctcagactggcattgcctttgttattggtccttgtagagagggtaattatctcaaagcaatcatgtaatcctcctcatttttcctttgaaagccttggtctccctttgcctccctgaatacgcacatagctgatcatggcaggtgtatcccactgcagtgctctacctccaaatagatatcgcggccgc

SEQ ID NO: 3 - DNA, 1280 bp, Artificial Sequence
  The sequence is synthetized.
  misc_feature (1)..(131): Homologous arm (homologous recombination for linking to 5'- terminal of mouse Ig γ1) (mouse sequence).
  misc_feature (132)..(176): Human Ig γ1 Hinge (human sequence).
  misc_feature (295)..(625): Human Ig γ1 CH2 (human sequence).
  misc_feature (722)..(1044): Human Ig γ1 CH3 (human sequence).
  misc_feature (1045)..(1280): Homologous arm (homologous recombination for linking to mouse Ig γ1 3'- terminal) (mouse sequence)
aaatgttggatatcacctactccatgtagagagtcggggacatgggaagggtgcaaaagagcggccttctagaaggtttggtcctgtcctgtcctgtctgacagtgtaatcacatatactttttcttgtagagcccaaatcttgtgacaaaactcacacatgcccaccgtgcccaggtaagccagcccaggcctcgccctccagctcaaggcgggacaggtgccctagagtagcctgcatccagggacaggccccagccgggtgctgacacgtccacctccatctcttcctcagcacctgaactcctggggggaccgtcagtcttcctcttccccccaaaacccaaggacaccctcatgatctcccggacccctgaggtcacatgcgtggtggtggacgtgagccacgaagaccctgaggtcaagttcaactggtacgtggacggcgtggaggtgcataatgccaagacaaagccgcgggaggagcagtacaacagcacgtaccgtgtggtcagcgtcctcaccgtcctgcaccaggactggctgaatggcaaggagtacaagtgcaaggtctccaacaaagccctcccagcccccatcgagaaaaccatctccaaagccaaaggtgggacccgtggggtgcgagggccacatggacagaggccggctcggcccaccctctgccctgagagtgaccgctgtaccaacctctgtccctacagggcagccccgagaaccacaggtgtacaccctgcccccatcccgggatgagctgaccaagaaccaggtcagcctgacctgcctggtcaaaggcttctatcccagcgacatcgccgtggagtgggagagcaatgggcagccggagaacaactacaagaccacgcctcccgtgctggactccgacggctccttcttcctctacagcaagctcaccgtggacaagagcaggtggcagcaggggaacgtcttctcatgctccgtgatgcatgaggctctgcacaaccactacacacagaagagcctctccctgtctccgggtaaatgatcccagtgtccttggagccctctggtcctacaggactctgacacctacctccacccctccctgtgtaaataaagcacccagcactgccttgggaccctgcaataatgtcctggtgatttctgagatgtagagtctagctaggtcatggaatgaggggtctccatggtttgaggcctgagttgtgactaaggaaaaacccataggcctacactgccacacccagcacttttgaattt